European Patent Application EP 4 332 218 A1, published March 6, 2024. Title: ONCOLYTIC VIRUS VECTOR AND APPLICATION THEREOF CROSS-REFERENCE TO RELATED APPLICATION. Applicant: SHANGHAI YUNYING BIOPHARMACEUTICAL TECHNOLOGY CO., LTD. Application PCT/CN2021/098139. The sequence listing filed with the application follows.

SEQUENCE LISTING (5 sequences)

SEQ ID NO: 1 - DNA, 718 bp, synthetic construct
ttaagatacattgatgagtttggacaaaccacaactagaatgcagtgaaaaaaatgctttatttgtgaaatttgtgatgctattgctttatttgtaaccattataagctgcaataaacaagtttcaggtttggaactggccggctggcctgggtgaggggctggggtgggctgtgggcacttctgcccttctctctgtcaccctcagttctgcccgcaggctctctttgatctgcgccttgggggccagggagatggccccacagaggtaggtgccgctgtcattgcgccgggccctgaccacgctcatgtggaagtcacgcccgttgggcagttgtgtgacacggaagcggcagtcctggccgggctggctgcggtcctcggggaaggcggccagcttgtccgtctggttgctggggctcattctataccagtttagcacgaagctctccgatgtgttggagaagctacaggtgaaggtggcgttgtccccttcggtcaccacgagcagggctggggagaaggtgggggggttccagggcctgtctggggagtctaagaaccatcctggccgccagcccagttgtagcaccgcccagacgactggccagggcgcctgtgggatctgcatctggagctagcgtctgaaacgagacgctaattagtgtatattttttcaattttaccggatatttatattccaaaaaaaaaaaataaaa

SEQ ID NO: 2 - DNA, 1432 bp, synthetic construct
cagagtgccagccctgggaccgaaccccgcgtttatgaacaaacgacccaacacccgtgcgttttattctgtctttttattgccgtcatagcgcgggttccttccggtattgtctccttccgtgtttcagttagcctcccccgtttaaactcattactaaccggtagggatcgaacccttttaaaaacatgtatcacttttgtcgcatgaagatgtcttcgaacttttaaaaacacgctgggcttcatcagatctttcaggtatatggattttttctcttttcttggtctgttcactctcttccctctccattgtgttggttccacatttataagagttgcgaggccgcttcttcttcttccatttccatagaattagacagaaaaccatcacacatataataactgttggaagtacagctgtaatccaaggaatgtggtctgggggaggctgagggtcctcaagctctatagagaaaggtgaagataaaagccgcgtcttgtcagtttccagaatacagaagatggtcatattgctcgtaacatcagggaatgaaacagacaagctgatggaaacgtcgtacagttctgtgacattatcttgagatttctgcataataccatcatactcgatagttgagttcttggttcttagcaaaacactcatcttcttaggttctgggtaaccgtgtatagatgagcaggtcaaatttatgtacacattttctgttatattagaaattggtactatttcaggttgactgaagttagcaagcactgacagttcagagttcatctggtggatgcgaatcattcctgtgggctttttgtgatggatgatacattgatacaagcccttgtccttgatctgaagattgtgaagtctcagggtccaactgtccgaatcaaaacttgtgcggcccatatacttggaatgaacactgtcaaatttctctttgcctaagtatacctcattcagaaccaagttttcctggtcctgccaaaatactactagctcactcaggctttggttttgagagtttgcaaattggcatggcaggtctgcagtctcattgaaataagcctgaatcttcagaggagcagcaccagagagcaggaaggccatcacaaagagaatgttactcagtcccatagtgcactggggatccatggtgcacaccaatgtggtgaatggtcaaatggcgtttattgtatcgagctaggcacttaaatacaatatctctgcaatgcgcaattcagtggttcgtccaatccatgtcagacccgtctgttgccttcctaataaggcacgatcgtaccaccttacttccaccaatcggcatgcacggtgctttttctctccttgtaaggcatgttgctaactcatcgttaccatgttgcaagactacaagagtattgcataagactacatt

SEQ ID NO: 3 - DNA, 2095 bp, synthetic construct
ggggggctataaaagggggtgggggcgttcgatgcggctctgcatcccgcaggtgctgttggccttgttcctttccatgctgacagggccgggagaaggcagctacccttacgatgtacctgattacgcccaagtgcagcttcagcagagcggcgctgagctggcccggcccggggcctctgtgaaaatgagctgcaaggcttccggttacacctttacaaggtacacaatgcactgggtgaagcagcggccagggcaggggctagagtggatcggctacataaacccatctcggggatatacaaactacaatcaaaagttcaaagacaaggccacactgacaacggacaagtcaagcagcacagcttacatgcaactgtcatctctgacatccgaggatagcgccgtttactattgcgccagatactatgatgaccactattgcttggactactggggacagggaacaaccctcacagttagctccggcggggggggcagtggaggtggaggatctgggggcggcggtagtcagatcgtcctcacacagtctccggccataatgtccgcctcccccggagagaaggttactatgacatgttccgcatcttcctctgtgtcatatatgaattggtatcagcagaagagtggcacctctcctaaacgctggatttacgatacctctaaactggcgtccggggtgcctgcacatttcagaggatcaggctccggtacgagttattcactcacaatatctggaatggaggccgaagatgccgctacttactactgccaacaatggtcaagcaaccccttcactttcgggagcgggacaaagctggagatcaacatggcctcctctgggtatgtcctccaggcggaactctccccctcaactgagaactcaagtcaactggacttcgaagatgtatggaactcttcctatggtgtgaatgattccttcccagatggagactatgatgccaacctggaagcagcagccccctgccactcctgtaacctgctggatgactctgcactgcccttcttcatcctcaccagtgtcctgggtatcctagctagcagcactgtcctcttcatgcttttcagacctctcttccgctggcagctctgccctggctggcctgtcctggcacaactggctgtgggcagtgccctcttcagcattgtggtgcccgtcttggccccagggctaggtagcactcgcagctctgccctgtgtagcctgggctactgtgtctggtatggctcagcctttgcccaggctttgctgctagggtgccatgcctccctgggccacagactgggtgcaggccaggtcccaggcctcaccctggggctcactgtgggaatttggggagtggctgccctactgacactgcctgtcaccctggccagtggtgcttctggtggactctgcaccctgatatacagcacggagctgaaggctttgcaggccacacacactgtagcctgtcttgccatctttgtcttgttgccattgggtttgtttggagccaaggggctgaagaaggcattgggtatggggccaggcccctggatgaatatcctgtgggcctggtttattttctggtggcctcatggggtggttctaggactggatttcctggtgaggtccaagctgttgctgttgtcaacatgtctggcccagcaggctctggacctgctgctgaacctggcagaagccctggcaattttgcactgtgtggctacgcccctgctcctcgccctattctgccaccaggccacccgcaccctcttgccctctctgcccctccctgaaggatggtcttctcatctggacacccttggaagcaaatcctaacgactgtgccttctagttgccagccatctgttgtttgcccctcccccgtgccttccttgaccctggaaggtgccactcccactgtcctttcctaataaaatgaggaaattgcatcgcattgtctgagtaggtgtcattctattctggggggtggggtggggcaggacagcaagggggaggattgggaagacaatagcaggaatgctggggatgcggtgggctctatgg

SEQ ID NO: 4 - DNA, 1247 bp, synthetic construct
ttctagagtcacgacgcatttgcccccgtccccgcagcaacacacaaagcgatttcaattttcacgattttattattaattacaccaaccaccctgtccccgggacgtggtcaggaccgggggtccgcacccaaacgcacgaaacaaatgctggcagtgtgccgaatataaccccgcgtaggaacacgtcgacgcgtgcgccaaacagcaccagaaggcgcatgccatcagcaggtcgtgcatatggcgatgtgtttggacgcagggcgcagccgcggcgataaaattcatggcggccgtccgccagggccacagcggcgaggactccctgttggcccgaagccattgggtatgaaccagctgcgcctcctgtccgaccctggctcccgccagcgggggcggtgggtcgtgggtgttgagagcacacaggcgggacacctcgatcaccgtccgaaaaaaggcccggtggtccgcgggcagcatctgcaggtgcgccagggcctgggcgttgagagggtacaactcggagccgggggactccgggggccggtccgcgcggtgccgcgagttggcacgctttggggcccgggtgtcggacgcgggcgcgttatggatcccgacgcggggcagaacgtacgtgcgttggcgcggcgatgaggggtccgggctgccgaggggggcgtaggggaccgggctaggcaagcccgcgggttgcgcggggttcccgtgggggtctaggctccctgggcacccgtgggggtcgtgggggtcgcgggtccctgggtatgcgcgggaccctgggttctctgggagatcgtggaactcgcggttccctgggctctcggggaacccggggctccctggggacacgtggtgccctgggaattcttgatggtcggacggcttcagatggcttcgggatcgagagggccgcacagactcgtagtagacccgaatctccacgtttccccgccgccggatcatggtcgccgccccggtgcgggggcccgtcggtcggaagcgagtgcccttcaagcgtgtccgctcctctgggctgcatgccgtcggatggggtgccttttaaggaaaggtctcggctgcccgccccaaccggggtttgggggtgggccggggaaaccccggatgccatggcattcgtttattacaagaattaaatcaagttggtatagtcttaaaactgcttgatcatgatcaacgtaataatcgccgtggatgtccattggtct

SEQ ID NO: 5 - DNA, 8734 bp, synthetic construct
ggaggaagggagggaggagggtactgggggtgaagaaggggggggggagaagcgagaacaggaaaggcgatggagcccggcagaacaccgaggaaaaaaaaaccacagcgcatgcgccgggccgttgtggggccccgggccggggccccttgggtccgccggggccccgggccgggccgccacgggggccggccgttggcggtaaccccgagtgttcatctcaggccccgggccgggaacccggaaaagcctccggggggcctttttcgcgtcgcgtgccggcgagcgggtccggacggggcccggaccgccgcggtcgggggcccctcgtcccgggccgtacgcggccttcgccccgtgaggggacagacgaacgaaacattccggcgacggaacgaaaaacaccccagacgggttaaagaaacagaaaccgcaacccccaccacccccgaaacggggaaaacgaaaaaacagaccagcggccggccggcgcttagggggaggatgtcgccgacgccccttggccgccccggctgcaggggggcccggagagccgcggcacccggacgcgcccggaaagtctttcgcaccacccgcgatcggcacggccgcgcccccgcttttataaaggctgagatgacgcagcaaaaacaggccacagcaccacgtgggtaggtgatgtaattttattttcctcgtctgcggcctaatggatttccgggcgcggtgcccctgtctgcagagcacttaacggaattctagagtcacgacgcatttgcccccgtccccgcagcaacacacaaagcgatttcaattttcacgattttattattaattacaccaaccaccctgtccccgggacgtggtcaggaccgggggtccgcacccaaacgcacgaaacaaatgctggcagtgtgccgaatataaccccgcgtaggaacacgtcgacgcgtgcgccaaacagcaccagaaggcgcatgccatcagcaggtcgtgcatatggcgatgtgtttggacgcagggcgcagccgcggcgataaaattcatggcggccgtccgccagggccacagcggcgaggactccctgttggcccgaagccattgggtatgaaccagctgcgcctcctgtccgaccctggctcccgccagcgggggcggtgggtcgtgggtgttgagagcacacaggcgggacacctcgatcaccgtccgaaaaaaggcccggtggtccgcgggcagcatctgcaggtgcgccagggcctgggcgttgagagggtacaactcggagccgggggactccgggggccggtccgcgcggtgccgcgagttggcacgctttggggcccgggtgtcggacgcgggcgcgttatggatcccgacgcggggcagaacgtacgtgcgttggcgcggcgatgaggggtccgggctgccgaggggggcgtaggggaccgggctaggcaagcccgcgggttgcgcggggttcccgtgggggtctaggctccctgggcacccgtgggggtcgtgggggtcgcgggtccctgggtatgcgcgggaccctgggttctctgggagatcgtggaactcgcggttccctgggctctcggggaacccggggctccctggggacacgtggtgccctgggaattcttgatggtcggacggcttcagatggcttcgggatcgagagggccgcacagactcgtagtagacccgaatctccacgtttccccgccgccggatcatggtcgccgccccggtgcgggggcccgtcggtcggaagcgagtgcccttcaagcgtgtccgctcctctgggctgcatgccgtcggatggggtgccttttaaggaaaggtctcggctgcccgccccaaccggggtttgggggtgggccggggaaaccccggatgccatggcattcgtttattacaagaattaaatcaagttggtatagtcttaaaactgcttgatcatgatcaacgtaataatcgccgtggatgtccattggtctaattcccatagagcccaccgcatccccagcattcctgctattgtcttcccaatcctcccccttgctgtcctgccccaccccaccccccagaatagaatgacacctactcagacaatgcgatgcaatttcctcattttattaggaaaggacagtgggagtggcaccttccagggtcaaggaaggcacgggggaggggcaaacaacagatggctggcaactagaaggcacagtcgttacttgtacagctcgtccatgccgagagtgatcccggcggcggtcacgaactccagcaggaccatgtgatcgcgcttctcgttggggtctttgctcagggcggactggtagctcaggtagtggttgtcgggcagcagcacggggccgtcgccgatgggggtgttctgctggtagtggtcggcgagctgcacgctgccgtcctcgatgttgtggcggatcttgaagttcaccttgatgccgttcttctgcttgtcggccatgatatagacgttgtggctgttgtagttgtactccagcttgtgccccaggatgttgccgtcctccttgaagtcgatgcccttcagctcgatgcggttcaccagggtgtcgccctcgaacttcacctcggcgcgggtcttgtagttgccgtcgtccttgaagaagatggtgcgctcctggacgtagccttcgggcatggcggacttgaagaagtcgtgctgcttcatgtggtcggggtagcgggcgaagcacttcaggccgtagccgaaggtggtcacgagggtgggccagggcacgggcagcttgccggtggtgcagatgaacttcagggtcagcttgccgtaggtggcatcgccctcgccctcgccggacacgctgaacttgtggccgtttacgtcgccgtccagctcgaccaggatgggcaccaccccggtgaacagctcctcgcccttgctcaccatctcaccatggtggcgtccggtagcgctagcggatctgacggttcactaaaccagctctgcttatatagacctcccaccgtacacgcctaccgcccatttgcgtcaatggggcggagttgttacgacattttggaaagtcccgttgattttggtgccaaaacaaactcccattgacgtcaatggggtggagacttggaaatccccgtgagtcaaaccgctatccacgcccattgatgtactgccaaaaccgcatcaccatggtaatagcgatgactaatacgtagatgtactgccaagtaggaaagtcccataaggtcatgtactgggcataatgccaggcgggccatttaccgtcattgacgtcaatagggggcgtacttggcatatgatacacttgatgtactgccaagtgggcagtttaccgtaaatactccacccattgacgtcaatggaaagtccctattggcgttactatgggaacatacgtcattattgacgtcaatgggcgggggtcgttgggcggtcagccaggcgggccatttaccgtaagttatgtaacgcggaactccatatatgggctatgaactaatgaccccgtaattgattactattaataactaatgcatggcggtaatacggttatccacgcggccgcctagcttgcatgcaggcctctgcagtcgacgggcccgggatccgattaagatacattgatgagtttggacaaaccacaactagaatgcagtgaaaaaaatgctttatttgtgaaatttgtgatgctattgctttatttgtaaccattataagctgcaataaacaagtttcaggtttggaactggccggctggcctgggtgaggggctggggtgggctgtgggcacttctgcccttctctctgtcaccctcagttctgcccgcaggctctctttgatctgcgccttgggggccagggagatggccccacagaggtaggtgccgctgtcattgcgccgggccctgaccacgctcatgtggaagtcacgcccgttgggcagttgtgtgacacggaagcggcagtcctggccgggctggctgcggtcctcggggaaggcggccagcttgtccgtctggttgctggggctcattctataccagtttagcacgaagctctccgatgtgttggagaagctacaggtgaaggtggcgttgtccccttcggtcaccacgagcagggctggggagaaggtgggggggttccagggcctgtctggggagtctaagaaccatcctggccgccagcccagttgtagcaccgcccagacgactggccagggcgcctgtgggatctgcatctggagctagcgtctgaaacgagacgctaattagtgtatattttttcaattttaccggatatttatattccaaaaaaaaaaaataaaaatctagatgcattcgcgaggtacccagagtgccagccctgggaccgaaccccgcgtttatgaacaaacgacccaacacccgtgcgttttattctgtctttttattgccgtcatagcgcgggttccttccggtattgtctccttccgtgtttcagttagcctcccccgtttaaactcattactaaccggtagggatcgaacccttttaaaaacatgtatcacttttgtcgcatgaagatgtcttcgaacttttaaaaacacgctgggcttcatcagatctttcaggtatatggattttttctcttttcttggtctgttcactctcttccctctccattgtgttggttccacatttataagagttgcgaggccgcttcttcttcttccatttccatagaattagacagaaaaccatcacacatataataactgttggaagtacagctgtaatccaaggaatgtggtctgggggaggctgagggtcctcaagctctatagagaaaggtgaagataaaagccgcgtcttgtcagtttccagaatacagaagatggtcatattgctcgtaacatcagggaatgaaacagacaagctgatggaaacgtcgtacagttctgtgacattatcttgagatttctgcataataccatcatactcgatagttgagttcttggttcttagcaaaacactcatcttcttaggttctgggtaaccgtgtatagatgagcaggtcaaatttatgtacacattttctgttatattagaaattggtactatttcaggttgactgaagttagcaagcactgacagttcagagttcatctggtggatgcgaatcattcctgtgggctttttgtgatggatgatacattgatacaagcccttgtccttgatctgaagattgtgaagtctcagggtccaactgtccgaatcaaaacttgtgcggcccatatacttggaatgaacactgtcaaatttctctttgcctaagtatacctcattcagaaccaagttttcctggtcctgccaaaatactactagctcactcaggctttggttttgagagtttgcaaattggcatggcaggtctgcagtctcattgaaataagcctgaatcttcagaggagcagcaccagagagcaggaaggccatcacaaagagaatgttactcagtcccatagtgcactggggatccatggtgcacaccaatgtggtgaatggtcaaatggcgtttattgtatcgagctaggcacttaaatacaatatctctgcaatgcgcaattcagtggttcgtccaatccatgtcagacccgtctgttgccttcctaataaggcacgatcgtaccaccttacttccaccaatcggcatgcacggtgctttttctctccttgtaaggcatgttgctaactcatcgttaccatgttgcaagactacaagagtattgcataagactacatttctagatggggggctataaaagggggtgggggcgttcgatgcggctctgcatcccgcaggtgctgttggccttgttcctttccatgctgacagggccgggagaaggcagctacccttacgatgtacctgattacgcccaagtgcagcttcagcagagcggcgctgagctggcccggcccggggcctctgtgaaaatgagctgcaaggcttccggttacacctttacaaggtacacaatgcactgggtgaagcagcggccagggcaggggctagagtggatcggctacataaacccatctcggggatatacaaactacaatcaaaagttcaaagacaaggccacactgacaacggacaagtcaagcagcacagcttacatgcaactgtcatctctgacatccgaggatagcgccgtttactattgcgccagatactatgatgaccactattgcttggactactggggacagggaacaaccctcacagttagctccggcggggggggcagtggaggtggaggatctgggggcggcggtagtcagatcgtcctcacacagtctccggccataatgtccgcctcccccggagagaaggttactatgacatgttccgcatcttcctctgtgtcatatatgaattggtatcagcagaagagtggcacctctcctaaacgctggatttacgatacctctaaactggcgtccggggtgcctgcacatttcagaggatcaggctccggtacgagttattcactcacaatatctggaatggaggccgaagatgccgctacttactactgccaacaatggtcaagcaaccccttcactttcgggagcgggacaaagctggagatcaacatggcctcctctgggtatgtcctccaggcggaactctccccctcaactgagaactcaagtcaactggacttcgaagatgtatggaactcttcctatggtgtgaatgattccttcccagatggagactatgatgccaacctggaagcagcagccccctgccactcctgtaacctgctggatgactctgcactgcccttcttcatcctcaccagtgtcctgggtatcctagctagcagcactgtcctcttcatgcttttcagacctctcttccgctggcagctctgccctggctggcctgtcctggcacaactggctgtgggcagtgccctcttcagcattgtggtgcccgtcttggccccagggctaggtagcactcgcagctctgccctgtgtagcctgggctactgtgtctggtatggctcagcctttgcccaggctttgctgctagggtgccatgcctccctgggccacagactgggtgcaggccaggtcccaggcctcaccctggggctcactgtgggaatttggggagtggctgccctactgacactgcctgtcaccctggccagtggtgcttctggtggactctgcaccctgatatacagcacggagctgaaggctttgcaggccacacacactgtagcctgtcttgccatctttgtcttgttgccattgggtttgtttggagccaaggggctgaagaaggcattgggtatggggccaggcccctggatgaatatcctgtgggcctggtttattttctggtggcctcatggggtggttctaggactggatttcctggtgaggtccaagctgttgctgttgtcaacatgtctggcccagcaggctctggacctgctgctgaacctggcagaagccctggcaattttgcactgtgtggctacgcccctgctcctcgccctattctgccaccaggccacccgcaccctcttgccctctctgcccctccctgaaggatggtcttctcatctggacacccttggaagcaaatcctaacgactgtgccttctagttgccagccatctgttgtttgcccctcccccgtgccttccttgaccctggaaggtgccactcccactgtcctttcctaataaaatgaggaaattgcatcgcattgtctgagtaggtgtcattctattctggggggtggggtggggcaggacagcaagggggaggattgggaagacaatagcaggaatgctggggatgcggtgggctctatggatcggatcccgggcccgtcgactgcagaggcctgcatgcaagcttgggagccagttagattgcatgtgatcgttgggaatgacccccggggttataaaaggcgcgtcccgtggacgcggccctcggttgggcgacgcatgccagcccaacaaaatccgccggggtgccagtcccattcccgaaggcgtagcccgttaacttggctggcttggatggggagtagggccttttccattaccccaaggacctagcgcgcgggagtcgtggctttggggcgcatccatggcttcggaggcggcgcaacccgacgcgggtttatggagcgcggggaacgcgtttgctgatcccccgcccccctacgatagcttgtctggtaggaacgaggggccgtttgtcgttattgatctggacacccccacggacccacctccaccgtactctgctgggcccctgttgtccgtgccaattccgccaacctcctccggagagggcgaggcgtcggagcggggccgctcacgccaagccgcccagcgagccgctcggcgcgcccggcgccgcgccgaacgacgtgcgcagcgccggagttttggccctggcgggttattggcaacccccctgtttcttccggaaaccaggcttgtggccccacccgacatcacaagggacctcttgtcgggcctcccgacgtacgccgaggctatgtcggaccaccccccaacctatgccactgtcgtggccgttcgttcgaccgaacagccgtccggggctttggcgcccgacgaccagcgacgaacgcaaaact